European Patent Specification EP 3 558 390 B1, published October 9, 2024. Title: NOVEL AMANITIN CONJUGATE. Applicant: Heidelberg Pharma Research GmbH. The sequence listing filed with the application follows.

SEQUENCE LISTING (2 sequences)

SEQ ID NO: 1 - protein, 450 aa, Artificial Sequence
  Humanized J22.9 heavy chain J22.9-ISY-D265C
EVQLVESGGGLVQPGGSLRLSCAASGFTFSRYWISWVRQAPGKGLVWVGEINPSSSTINYAPSLKDKFTISRDNAKNTLYLQMNSLRAEDTAVYYCASLYYDYGDAYDYWGQGTLVTVSSASTKGPSVFPLAPSSKSTSGGTAALGCLVKDYFPEPVTVSWNSGALTSGVHTFPAVLQSSGLYSLSSVVTVPSSSLGTQTYICNVNHKPSNTKVDKKVEPKSCDKTHTCPPCPAPELLGGPSVFLFPPKPKDTLMISRTPEVTCVVVCVSHEDPEVKFNWYVDGVEVHNAKTKPREEQYNSTYRVVSVLTVLHQDWLNGKEYKCKVSNKALPAPIEKTISKAKGQPREPQVYTLPPSREEMTKNQVSLTCLVKGFYPSDIAVEWESNGQPENNYKTTPPVLDSDGSFFLYSKLTVDKSRWQQGNVFSCSVMHEALHNHYTQKSLSLSPGK

SEQ ID NO: 2 - protein, 214 aa, Artificial Sequence
  Humanized J22.9 light chain
EIVMTQSPATLSVSPGERATLSCKASQSVESNVAWYQQKPGQAPRALIYSASLRFSGIPARFSGSGSGTEFTLTISSLQSEDFAVYYCQQYNNYPLTFGAGTKLELKRTVAAPSVFIFPPSDEQLKSGTASVVCLLNNFYPREAKVQWKVDNALQSGNSQESVTEQDSKDSTYSLSSTLTLSKADYEKHKVYACEVTHQGLSSPVTKSFNRGEC